European Patent Specification EP 3 913 001 B1, published September 11, 2024. Title: ANTI-CLD18A2 NANOBODY AND APPLICATION THEREOF. Applicant: ZHEJIANG DOER BIOLOGICS CORPORATION. The sequence listing filed with the application follows.

SEQUENCE LISTING (144 sequences)

SEQ ID NO: 1 - protein, 25 aa, Artificial Sequence
  Amino acid sequence of FR1
QLQLVESGGGLVQPGGSLRLSCAAS

SEQ ID NO: 2 - protein, 25 aa, Artificial Sequence
  Amino acid sequence of FR1
QVQLVESGGGLVQPGGSLRLSCAAS

SEQ ID NO: 3 - protein, 25 aa, Artificial Sequence
  Amino acid sequence of FR1
QVQLVESGGGLVQPGGSLRLSCTAS

SEQ ID NO: 4 - protein, 8 aa, Artificial Sequence
  Amino acid sequence of CDR1
GGIFSIGV

SEQ ID NO: 5 - protein, 8 aa, Artificial Sequence
  Amino acid sequence of CDR1
GSIFLINA

SEQ ID NO: 6 - protein, 8 aa, Artificial Sequence
  Amino acid sequence of CDR1
GSIFRIDG

SEQ ID NO: 7 - protein, 8 aa, Artificial Sequence
  Amino acid sequence of CDR1
GVDISSDV

SEQ ID NO: 8 - protein, 8 aa, Artificial Sequence
  Amino acid sequence of CDR1
GSIFSINA

SEQ ID NO: 9 - protein, 8 aa, Artificial Sequence
  Amino acid sequence of CDR1
GSIFMINV

SEQ ID NO: 10 - protein, 7 aa, Artificial Sequence
  Amino acid sequence of CDR1
GEISSDA

SEQ ID NO: 11 - protein, 8 aa, Artificial Sequence
  Amino acid sequence of CDR1
GSIFSIPV

SEQ ID NO: 12 - protein, 17 aa, Artificial Sequence
  Amino acid sequence of FR2
MGWYRQAPGKQRELVAT

SEQ ID NO: 13 - protein, 17 aa, Artificial Sequence
  Amino acid sequence of FR2
MGWYRQAPGKQRELVAV

SEQ ID NO: 14 - protein, 17 aa, Artificial Sequence
  Amino acid sequence of FR2
MHWYRQAPGKQRELVAS

SEQ ID NO: 15 - protein, 17 aa, Artificial Sequence
  Amino acid sequence of FR2
MAWYRQAPGKQREFVSG

SEQ ID NO: 16 - protein, 17 aa, Artificial Sequence
  Amino acid sequence of FR2
MGWYRQAPGKQRELVAA

SEQ ID NO: 17 - protein, 17 aa, Artificial Sequence
  Amino acid sequence of FR2
MAWYRQAPGKQRELVAG

SEQ ID NO: 18 - protein, 17 aa, Artificial Sequence
  Amino acid sequence of FR2
MTWYRQALGKEREFVAG

SEQ ID NO: 19 - protein, 7 aa, Artificial Sequence
  Amino acid sequence of CDR2
ITSRGST

SEQ ID NO: 20 - protein, 7 aa, Artificial Sequence
  Amino acid sequence of CDR2
ITRGGSA

SEQ ID NO: 21 - protein, 7 aa, Artificial Sequence
  Amino acid sequence of CDR2
ITPSGIT

SEQ ID NO: 22 - protein, 7 aa, Artificial Sequence
  Amino acid sequence of CDR2
LTRGGSI

SEQ ID NO: 23 - protein, 8 aa, Artificial Sequence
  Amino acid sequence of CDR2
ITFGGGST

SEQ ID NO: 24 - protein, 7 aa, Artificial Sequence
  Amino acid sequence of CDR2
ITRGAST

SEQ ID NO: 25 - protein, 7 aa, Artificial Sequence
  Amino acid sequence of CDR2
MTRGGST

SEQ ID NO: 26 - protein, 7 aa, Artificial Sequence
  Amino acid sequence of CDR2
ISKGGTS

SEQ ID NO: 27 - protein, 38 aa, Artificial Sequence
  Amino acid sequence of FR3
NYADSVKGRFTISGDNAKNTVYLQMNNLKPEDTAVYYC

SEQ ID NO: 28 - protein, 38 aa, Artificial Sequence
  Amino acid sequence of FR3
NYTDSVKGRFTISRDNAKNTVYLQMNSLKPEDTAVYYC

SEQ ID NO: 29 - protein, 38 aa, Artificial Sequence
  Amino acid sequence of FR3
HYADSVKGRFTISRDIAKKMQYLQMNSLKPEDTAVYYC

SEQ ID NO: 30 - protein, 38 aa, Artificial Sequence
  Amino acid sequence of FR3
NYADSVKGRFTISRDFAKNTVDLQMNSLKPEDTAVYYC

SEQ ID NO: 31 - protein, 38 aa, Artificial Sequence
  Amino acid sequence of FR3
NYADSVKGRFTISRDNAKNTVYLQMNSLKPEDTAVYYC

SEQ ID NO: 32 - protein, 38 aa, Artificial Sequence
  Amino acid sequence of FR3
NYADSVKGRFTVSRDNAKNTVYLQMNSLKSEDTAVYYC

SEQ ID NO: 33 - protein, 15 aa, Artificial Sequence
  Amino acid sequence of CDR3
YADLIRPGDFYGMDY

SEQ ID NO: 34 - protein, 16 aa, Artificial Sequence
  Amino acid sequence of CDR3
NADLNLRSDPFKWYTF

SEQ ID NO: 35 - protein, 15 aa, Artificial Sequence
  Amino acid sequence of CDR3
NAHLVKVGGVWSDEY

SEQ ID NO: 36 - protein, 14 aa, Artificial Sequence
  Amino acid sequence of CDR3
NAEIYTGTFYPRSY

SEQ ID NO: 37 - protein, 15 aa, Artificial Sequence
  Amino acid sequence of CDR3
NADLLVGGFPRRNVY

SEQ ID NO: 38 - protein, 16 aa, Artificial Sequence
  Amino acid sequence of CDR3
NADLNLASDPFKWYTY

SEQ ID NO: 39 - protein, 15 aa, Artificial Sequence
  Amino acid sequence of CDR3
NAQASSFGWMPLSDY

SEQ ID NO: 40 - protein, 11 aa, Artificial Sequence
  Amino acid sequence of FR4
WGKGTLVTVSS

SEQ ID NO: 41 - protein, 11 aa, Artificial Sequence
  Amino acid sequence of FR4
WGQGTQVTVSS

SEQ ID NO: 42 - protein, 121 aa, Artificial Sequence
  Amino acid sequence of the anti-CLD18A2 nanobody
QLQLVESGGGLVQPGGSLRLSCAASGGIFSIGVMGWYRQAPGKQRELVATITSRGSTNYADSVKGRFTISGDNAKNTVYLQMNNLKPEDTAVYYCYADLIRPGDFYGMDYWGKGTLVTVSS

SEQ ID NO: 43 - protein, 122 aa, Artificial Sequence
  Amino acid sequence of the anti-CLD18A2 nanobody
QVQLVESGGGLVQPGGSLRLSCAASGSIFLINAMGWYRQAPGKQRELVAVITRGGSANYTDSVKGRFTISRDNAKNTVYLQMNSLKPEDTAVYYCNADLNLRSDPFKWYTFWGQGTQVTVSS

SEQ ID NO: 44 - protein, 121 aa, Artificial Sequence
  Amino acid sequence of the anti-CLD18A2 nanobody
QVQLVESGGGLVQPGGSLRLSCTASGSIFRIDGMHWYRQAPGKQRELVASITPSGITHYADSVKGRFTISRDIAKKMQYLQMNSLKPEDTAVYYCNAHLVKVGGVWSDEYWGQGTQVTVSS

SEQ ID NO: 45 - protein, 120 aa, Artificial Sequence
  Amino acid sequence of the anti-CLD18A2 nanobody
QLQLVESGGGLVQPGGSLRLSCAASGVDISSDVMAWYRQAPGKQREFVSGLTRGGSINYADSVKGRFTISRDFAKNTVDLQMNSLKPEDTAVYYCNAEIYTGTFYPRSYWGQGTQVTVSS

SEQ ID NO: 46 - protein, 122 aa, Artificial Sequence
  Amino acid sequence of the anti-CLD18A2 nanobody
QVQLVESGGGLVQPGGSLRLSCAASGSIFSINAMGWYRQAPGKQRELVAAITFGGGSTNYADSVKGRFTISRDNAKNTVYLQMNSLKPEDTAVYYCNADLLVGGFPRRNVYWGQGTQVTVSS

SEQ ID NO: 47 - protein, 122 aa, Artificial Sequence
  Amino acid sequence of the anti-CLD18A2 nanobody
QVQLVESGGGLVQPGGSLRLSCAASGSIFMINVMGWYRQAPGKQRELVAVITRGASTNYADSVKGRFTISRDNAKNTVYLQMNSLKPEDTAVYYCNADLNLASDPFKWYTYWGQGTQVTVSS

SEQ ID NO: 48 - protein, 119 aa, Artificial Sequence
  Amino acid sequence of the anti-CLD18A2 nanobody
QLQLVESGGGLVQPGGSLRLSCAASGEISSDAMAWYRQAPGKQRELVAGMTRGGSTNYADSVKGRFTISRDFAKNTVDLQMNSLKPEDTAVYYCNAEIYTGTFYPRSYWGQGTQVTVSS

SEQ ID NO: 49 - protein, 121 aa, Artificial Sequence
  Amino acid sequence of the anti-CLD18A2 nanobody
QVQLVESGGGLVQPGGSLRLSCAASGSIFSIPVMTWYRQALGKEREFVAGISKGGTSNYADSVKGRFTVSRDNAKNTVYLQMNSLKSEDTAVYYCNAQASSFGWMPLSDYWGQGTQVTVSS

SEQ ID NO: 50 - protein, 17 aa, Artificial Sequence
  Amino acid sequence
MGWVRQAPGKGLEWVAT

SEQ ID NO: 51 - protein, 17 aa, Artificial Sequence
  Amino acid sequence
MGWYRQAPGKGLELVAT

SEQ ID NO: 52 - protein, 38 aa, Artificial Sequence
  Amino acid sequence
NYADSVKGRFTISRDNSKNTLYLQMNSLRAEDTAVYYC

SEQ ID NO: 53 - protein, 38 aa, Artificial Sequence
  Amino acid sequence
HYADSVKGRFTISRDNSKNTLYLQMNSLRAEDTAVYYC

SEQ ID NO: 54 - protein, 11 aa, Artificial Sequence
  Amino acid sequence
WGQGTLVTVSS

SEQ ID NO: 55 - protein, 17 aa, Artificial Sequence
  Amino acid sequence
MGWVRQAPGKGLEWVAV

SEQ ID NO: 56 - protein, 17 aa, Artificial Sequence
  Amino acid sequence
MHWVRQAPGKGLEWVAS

SEQ ID NO: 57 - protein, 17 aa, Artificial Sequence
  Amino acid sequence
MAWVRQAPGKGLEWVSG

SEQ ID NO: 58 - protein, 17 aa, Artificial Sequence
  Amino acid sequence
MGWVRQAPGKGLEWVAA

SEQ ID NO: 59 - protein, 17 aa, Artificial Sequence
  Amino acid sequence
MAWVRQAPGKGLEWVAG

SEQ ID NO: 60 - protein, 17 aa, Artificial Sequence
  Amino acid sequence
MTWVRQAPGKGLEWVAG

SEQ ID NO: 61 - protein, 17 aa, Artificial Sequence
  Amino acid sequence
MGWYRQAPGKGLELVAV

SEQ ID NO: 62 - protein, 17 aa, Artificial Sequence
  Amino acid sequence
MHWYRQAPGKGLELVAS

SEQ ID NO: 63 - protein, 17 aa, Artificial Sequence
  Amino acid sequence
MAWYRQAPGKGLEFVSG

SEQ ID NO: 64 - protein, 17 aa, Artificial Sequence
  Amino acid sequence
MGWYRQAPGKGLELVAA

SEQ ID NO: 65 - protein, 17 aa, Artificial Sequence
  Amino acid sequence
MAWYRQAPGKGLELVAG

SEQ ID NO: 66 - protein, 17 aa, Artificial Sequence
  Amino acid sequence
MTWYRQAPGKGLEFVAG

SEQ ID NO: 67 - protein, 121 aa, Artificial Sequence
  Amino acid sequence of the anti-CLD18A2 nanobody
QVQLVESGGGLVQPGGSLRLSCAASGGIFSIGVMGWYRQAPGKQRELVATITSRGSTNYADSVKGRFTISRDNSKNTLYLQMNSLRAEDTAVYYCYADLIRPGDFYGMDYWGQGTLVTVSS

SEQ ID NO: 68 - protein, 122 aa, Artificial Sequence
  Amino acid sequence of the anti-CLD18A2 nanobody
QVQLVESGGGLVQPGGSLRLSCAASGSIFLINAMGWYRQAPGKQRELVAVITRGGSANYADSVKGRFTISRDNSKNTLYLQMNSLRAEDTAVYYCNADLNLRSDPFKWYTFWGQGTLVTVSS

SEQ ID NO: 69 - protein, 121 aa, Artificial Sequence
  Amino acid sequence of the anti-CLD18A2 nanobody
QVQLVESGGGLVQPGGSLRLSCAASGSIFRIDGMHWYRQAPGKQRELVASITPSGITHYADSVKGRFTISRDNSKNTLYLQMNSLRAEDTAVYYCNAHLVKVGGVWSDEYWGQGTLVTVSS

SEQ ID NO: 70 - protein, 120 aa, Artificial Sequence
  Amino acid sequence of the anti-CLD18A2 nanobody
QVQLVESGGGLVQPGGSLRLSCAASGVDISSDVMAWYRQAPGKQREFVSGLTRGGSINYADSVKGRFTISRDNSKNTLYLQMNSLRAEDTAVYYCNAEIYTGTFYPRSYWGQGTLVTVSS

SEQ ID NO: 71 - protein, 122 aa, Artificial Sequence
  Amino acid sequence of the anti-CLD18A2 nanobody
QVQLVESGGGLVQPGGSLRLSCAASGSIFSINAMGWYRQAPGKQRELVAAITFGGGSTNYADSVKGRFTISRDNSKNTLYLQMNSLRAEDTAVYYCNADLLVGGFPRRNVYWGQGTLVTVSS

SEQ ID NO: 72 - protein, 122 aa, Artificial Sequence
  Amino acid sequence of the anti-CLD18A2 nanobody
QVQLVESGGGLVQPGGSLRLSCAASGSIFMINVMGWYRQAPGKQRELVAVITRGASTNYADSVKGRFTISRDNSKNTLYLQMNSLRAEDTAVYYCNADLNLASDPFKWYTYWGQGTLVTVSS

SEQ ID NO: 73 - protein, 119 aa, Artificial Sequence
  Amino acid sequence of the anti-CLD18A2 nanobody
QVQLVESGGGLVQPGGSLRLSCAASGEISSDAMAWYRQAPGKQRELVAGMTRGGSTNYADSVKGRFTISRDNSKNTLYLQMNSLRAEDTAVYYCNAEIYTGTFYPRSYWGQGTLVTVSS

SEQ ID NO: 74 - protein, 121 aa, Artificial Sequence
  Amino acid sequence of the anti-CLD18A2 nanobody
QVQLVESGGGLVQPGGSLRLSCAASGSIFSIPVMTWYRQALGKEREFVAGISKGGTSNYADSVKGRFTISRDNSKNTLYLQMNSLRAEDTAVYYCNAQASSFGWMPLSDYWGQGTLVTVSS

SEQ ID NO: 75 - protein, 121 aa, Artificial Sequence
  Amino acid sequence of the anti-CLD18A2 nanobody
QVQLVESGGGLVQPGGSLRLSCAASGGIFSIGVMGWVRQAPGKGLEWVATITSRGSTNYADSVKGRFTISRDNSKNTLYLQMNSLRAEDTAVYYCYADLIRPGDFYGMDYWGQGTLVTVSS

SEQ ID NO: 76 - protein, 122 aa, Artificial Sequence
  Amino acid sequence of the anti-CLD18A2 nanobody
QVQLVESGGGLVQPGGSLRLSCAASGSIFLINAMGWVRQAPGKGLEWVAVITRGGSANYADSVKGRFTISRDNSKNTLYLQMNSLRAEDTAVYYCNADLNLRSDPFKWYTFWGQGTLVTVSS

SEQ ID NO: 77 - protein, 121 aa, Artificial Sequence
  Amino acid sequence of the anti-CLD18A2 nanobody
QVQLVESGGGLVQPGGSLRLSCAASGSIFRIDGMHWVRQAPGKGLEWVASITPSGITHYADSVKGRFTISRDNSKNTLYLQMNSLRAEDTAVYYCNAHLVKVGGVWSDEYWGQGTLVTVSS

SEQ ID NO: 78 - protein, 120 aa, Artificial Sequence
  Amino acid sequence of the anti-CLD18A2 nanobody
QVQLVESGGGLVQPGGSLRLSCAASGVDISSDVMAWVRQAPGKGLEWVSGLTRGGSINYADSVKGRFTISRDNSKNTLYLQMNSLRAEDTAVYYCNAEIYTGTFYPRSYWGQGTLVTVSS

SEQ ID NO: 79 - protein, 122 aa, Artificial Sequence
  Amino acid sequence of the anti-CLD18A2 nanobody
QVQLVESGGGLVQPGGSLRLSCAASGSIFSINAMGWVRQAPGKGLEWVAAITFGGGSTNYADSVKGRFTISRDNSKNTLYLQMNSLRAEDTAVYYCNADLLVGGFPRRNVYWGQGTLVTVSS

SEQ ID NO: 80 - protein, 122 aa, Artificial Sequence
  Amino acid sequence of the anti-CLD18A2 nanobody
QVQLVESGGGLVQPGGSLRLSCAASGSIFMINVMGWVRQAPGKGLEWVAVITRGASTNYADSVKGRFTISRDNSKNTLYLQMNSLRAEDTAVYYCNADLNLASDPFKWYTYWGQGTLVTVSS

SEQ ID NO: 81 - protein, 119 aa, Artificial Sequence
  Amino acid sequence of the anti-CLD18A2 nanobody
QVQLVESGGGLVQPGGSLRLSCAASGEISSDAMAWVRQAPGKGLEWVAGMTRGGSTNYADSVKGRFTISRDNSKNTLYLQMNSLRAEDTAVYYCNAEIYTGTFYPRSYWGQGTLVTVSS

SEQ ID NO: 82 - protein, 121 aa, Artificial Sequence
  Amino acid sequence of the anti-CLD18A2 nanobody
QVQLVESGGGLVQPGGSLRLSCAASGSIFSIPVMTWVRQAPGKGLEWVAGISKGGTSNYADSVKGRFTISRDNSKNTLYLQMNSLRAEDTAVYYCNAQASSFGWMPLSDYWGQGTLVTVSS

SEQ ID NO: 83 - protein, 121 aa, Artificial Sequence
  Amino acid sequence of the anti-CLD18A2 nanobody
QVQLVESGGGLVQPGGSLRLSCAASGGIFSIGVMGWYRQAPGKGLELVATITSRGSTNYADSVKGRFTISRDNSKNTLYLQMNSLRAEDTAVYYCYADLIRPGDFYGMDYWGQGTLVTVSS

SEQ ID NO: 84 - protein, 122 aa, Artificial Sequence
  Amino acid sequence of the anti-CLD18A2 nanobody
QVQLVESGGGLVQPGGSLRLSCAASGSIFLINAMGWYRQAPGKGLELVAVITRGGSANYADSVKGRFTISRDNSKNTLYLQMNSLRAEDTAVYYCNADLNLRSDPFKWYTFWGQGTLVTVSS

SEQ ID NO: 85 - protein, 121 aa, Artificial Sequence
  Amino acid sequence of the anti-CLD18A2 nanobody
QVQLVESGGGLVQPGGSLRLSCAASGSIFRIDGMHWYRQAPGKGLELVASITPSGITHYADSVKGRFTISRDNSKNTLYLQMNSLRAEDTAVYYCNAHLVKVGGVWSDEYWGQGTLVTVSS

SEQ ID NO: 86 - protein, 120 aa, Artificial Sequence
  Amino acid sequence of the anti-CLD18A2 nanobody
QVQLVESGGGLVQPGGSLRLSCAASGVDISSDVMAWYRQAPGKGLEFVSGLTRGGSINYADSVKGRFTISRDNSKNTLYLQMNSLRAEDTAVYYCNAEIYTGTFYPRSYWGQGTLVTVSS

SEQ ID NO: 87 - protein, 122 aa, Artificial Sequence
  Amino acid sequence of the anti-CLD18A2 nanobody
QVQLVESGGGLVQPGGSLRLSCAASGSIFSINAMGWYRQAPGKGLELVAAITFGGGSTNYADSVKGRFTISRDNSKNTLYLQMNSLRAEDTAVYYCNADLLVGGFPRRNVYWGQGTLVTVSS

SEQ ID NO: 88 - protein, 122 aa, Artificial Sequence
  Amino acid sequence of the anti-CLD18A2 nanobody
QVQLVESGGGLVQPGGSLRLSCAASGSIFMINVMGWYRQAPGKGLELVAVITRGASTNYADSVKGRFTISRDNSKNTLYLQMNSLRAEDTAVYYCNADLNLASDPFKWYTYWGQGTLVTVSS

SEQ ID NO: 89 - protein, 119 aa, Artificial Sequence
  Amino acid sequence of the anti-CLD18A2 nanobody
QVQLVESGGGLVQPGGSLRLSCAASGEISSDAMAWYRQAPGKGLELVAGMTRGGSTNYADSVKGRFTISRDNSKNTLYLQMNSLRAEDTAVYYCNAEIYTGTFYPRSYWGQGTLVTVSS

SEQ ID NO: 90 - protein, 121 aa, Artificial Sequence
  Amino acid sequence of the anti-CLD18A2 nanobody
QVQLVESGGGLVQPGGSLRLSCAASGSIFSIPVMTWYRQAPGKGLEFVAGISKGGTSNYADSVKGRFTISRDNSKNTLYLQMNSLRAEDTAVYYCNAQASSFGWMPLSDYWGQGTLVTVSS

SEQ ID NO: 91 - protein, 231 aa, Artificial Sequence
  Amino acid sequence of the immunoglobulin Fc region
EPKSCDKTHTCPPCPAPELLGGPSVFLFPPKPKDTLMISRTPEVTCVVVDVSHEDPEVKFNWYVDGVEVHNAKTKPREEQYNSTYRVVSVLTVLHQDWLNGKEYKCKVSNKALPAPIEKTISKAKGQPREPQVYTLPPSRDELTKNQVSLTCLVKGFYPSDIAVEWESNGQPENNYKTTPPVLDSDGSFFLYSKLTVDKSRWQQGNVFSCSVMHEALHNHYTQKSLSLSPG

SEQ ID NO: 92 - protein, 231 aa, Artificial Sequence; identical to SEQ ID NO: 91
  Amino acid sequence of the immunoglobulin Fc region

SEQ ID NO: 93 - protein, 226 aa, Artificial Sequence
  Amino acid sequence of the immunoglobulin Fc region
DKTHTCPPCPAPELLGGPSVFLFPPKPKDTLMISRTPEVTCVVVDVSHEDPEVKFNWYVDGVEVHNAKTKPREEQYNSTYRVVSVLTVLHQDWLNGKEYKCKVSNKALPAPIEKTISKAKGQPREPQVYTLPPSRDELTKNQVSLTCLVKGFYPSDIAVEWESNGQPENNYKTTPPVLDSDGSFFLYSKLTVDKSRWQQGNVFSCSVMHEALHNHYTQKSLSLSPG

SEQ ID NO: 94 - protein, 231 aa, Artificial Sequence
  Amino acid sequence of the immunoglobulin Fc region
EPKSCDKTHTCPPCPAPELLGGPDVFLFPPKPKDTLMISRTPEVTCVVVDVSHEDPEVKFNWYVDGVEVHNAKTKPREEQYNSTYRVVSVLTVLHQDWLNGKEYKCKVSNKALPAPEEKTISKAKGQPREPQVYTLPPSRDELTKNQVSLTCLVKGFYPSDIAVEWESNGQPENNYKTTPPVLDSDGSFFLYSKLTVDKSRWQQGNVFSCSVMHEALHNHYTQKSLSLSPG

SEQ ID NO: 95 - protein, 231 aa, Artificial Sequence
  Amino acid sequence of the immunoglobulin Fc region
EPKSCDKTHTCPPCPAPELLGGPSVFLFPPKPKDTLMISRTPEVTCVVVDVSHEDPEVKFNWYVDGVEVHNAKTKPREEQYNSTYRVVSVLTVLHQDWLNGKEYKCKVSNWALPAPISKTISKAKGQPREPQVYTLPPSRDELTKNQVSLTCLVKGFYPSDIAVEWESNGQPENNYKTTPPVLDSDGSFFLYSKLTVDKSRWQQGNVFSCSVMHEALHNHYTQKSLSLSPG

SEQ ID NO: 96 - protein, 261 aa, Artificial Sequence
  Amino acid sequence of CLD18A1
MSTTTCQVVAFLLSILGLAGCIAATGMDMWSTQDLYDNPVTSVFQYEGLWRSCVRQSSGFTECRPYFTILGLPAMLQAVRALMIVGIVLGAIGLLVSIFALKCIRIGSMEDSAKANMTLTSGIMFIVSGLCAIAGVSVFANMLVTNFWMSTANMYTGMGGMVQTVQTRYTFGAALFVGWVAGGLTLIGGVMMCIACRGLAPEETNYKAVSYHASGHSVAYKPGGFKASTGFGSNTKNKKIYDGGARTEDEVQSYPSKHDYV

SEQ ID NO: 97 - protein, 261 aa, Artificial Sequence
  Amino acid sequence of CLD18A2
MAVTACQGLGFVVSLIGIAGIIAATCMDQWSTQDLYNNPVTAVFNYQGLWRSCVRESSGFTECRGYFTLLGLPAMLQAVRALMIVGIVLGAIGLLVSIFALKCIRIGSMEDSAKANMTLTSGIMFIVSGLCAIAGVSVFANMLVTNFWMSTANMYTGMGGMVQTVQTRYTFGAALFVGWVAGGLTLIGGVMMCIACRGLAPEETNYKAVSYHASGHSVAYKPGGFKASTGFGSNTKNKKIYDGGARTEDEVQSYPSKHDYV

SEQ ID NO: 98 - protein, 352 aa, Artificial Sequence
  Amino acid sequence of Anti-C18.2-6-Fc
QVQLVESGGGLVQPGGSLRLSCAASGGIFSIGVMGWYRQAPGKQRELVATITSRGSTNYADSVKGRFTISGDNAKNTVYLQMNNLKPEDTAVYYCYADLIRPGDFYGMDYWGQGTLVTVSSEPKSCDKTHTCPPCPAPELLGGPSVFLFPPKPKDTLMISRTPEVTCVVVDVSHEDPEVKFNWYVDGVEVHNAKTKPREEQYNSTYRVVSVLTVLHQDWLNGKEYKCKVSNKALPAPIEKTISKAKGQPREPQVYTLPPSRDELTKNQVSLTCLVKGFYPSDIAVEWESNGQPENNYKTTPPVLDSDGSFFLYSKLTVDKSRWQQGNVFSCSVMHEALHNHYTQKSLSLSPG

SEQ ID NO: 99 - protein, 353 aa, Artificial Sequence
  Amino acid sequence of Anti-C18.2-7-Fc
QVQLVESGGGLVQPGGSLRLSCAASGSIFLINAMGWYRQAPGKQRELVAVITRGGSANYTDSVKGRFTISRDNAKNTVYLQMNSLKPEDTAVYYCNADLNLRSDPFKWYTFWGQGTLVTVSSEPKSCDKTHTCPPCPAPELLGGPSVFLFPPKPKDTLMISRTPEVTCVVVDVSHEDPEVKFNWYVDGVEVHNAKTKPREEQYNSTYRVVSVLTVLHQDWLNGKEYKCKVSNKALPAPIEKTISKAKGQPREPQVYTLPPSRDELTKNQVSLTCLVKGFYPSDIAVEWESNGQPENNYKTTPPVLDSDGSFFLYSKLTVDKSRWQQGNVFSCSVMHEALHNHYTQKSLSLSPG

SEQ ID NO: 100 - protein, 352 aa, Artificial Sequence
  Amino acid sequence of Anti-C18.2-15-Fc
QVQLVESGGGLVQPGGSLRLSCTASGSIFRIDGMHWYRQAPGKQRELVASITPSGITHYADSVKGRFTISRDIAKKMQYLQMNSLKPEDTAVYYCNAHLVKVGGVWSDEYWGQGTLVTVSSEPKSCDKTHTCPPCPAPELLGGPSVFLFPPKPKDTLMISRTPEVTCVVVDVSHEDPEVKFNWYVDGVEVHNAKTKPREEQYNSTYRVVSVLTVLHQDWLNGKEYKCKVSNKALPAPIEKTISKAKGQPREPQVYTLPPSRDELTKNQVSLTCLVKGFYPSDIAVEWESNGQPENNYKTTPPVLDSDGSFFLYSKLTVDKSRWQQGNVFSCSVMHEALHNHYTQKSLSLSPG

SEQ ID NO: 101 - protein, 351 aa, Artificial Sequence
  Amino acid sequence of Anti-C18.2-19-Fc
QVQLVESGGGLVQPGGSLRLSCAASGVDISSDVMAWYRQAPGKQREFVSGLTRGGSINYADSVKGRFTISRDFAKNTVDLQMNSLKPEDTAVYYCNAEIYTGTFYPRSYWGQGTLVTVSSEPKSCDKTHTCPPCPAPELLGGPSVFLFPPKPKDTLMISRTPEVTCVVVDVSHEDPEVKFNWYVDGVEVHNAKTKPREEQYNSTYRVVSVLTVLHQDWLNGKEYKCKVSNKALPAPIEKTISKAKGQPREPQVYTLPPSRDELTKNQVSLTCLVKGFYPSDIAVEWESNGQPENNYKTTPPVLDSDGSFFLYSKLTVDKSRWQQGNVFSCSVMHEALHNHYTQKSLSLSPG

SEQ ID NO: 102 - protein, 353 aa, Artificial Sequence
  amino acid sequence of Anti-C18.2-20-Fc
QVQLVESGGGLVQPGGSLRLSCAASGSIFSINAMGWYRQAPGKQRELVAAITFGGGSTNYADSVKGRFTISRDNAKNTVYLQMNSLKPEDTAVYYCNADLLVGGFPRRNVYWGQGTLVTVSSEPKSCDKTHTCPPCPAPELLGGPSVFLFPPKPKDTLMISRTPEVTCVVVDVSHEDPEVKFNWYVDGVEVHNAKTKPREEQYNSTYRVVSVLTVLHQDWLNGKEYKCKVSNKALPAPIEKTISKAKGQPREPQVYTLPPSRDELTKNQVSLTCLVKGFYPSDIAVEWESNGQPENNYKTTPPVLDSDGSFFLYSKLTVDKSRWQQGNVFSCSVMHEALHNHYTQKSLSLSPG

SEQ ID NO: 103 - protein, 353 aa, Artificial Sequence
  Amino acid sequence of Anti-C18.2-28-Fc
QVQLVESGGGLVQPGGSLRLSCAASGSIFMINVMGWYRQAPGKQRELVAVITRGASTNYADSVKGRFTISRDNAKNTVYLQMNSLKPEDTAVYYCNADLNLASDPFKWYTYWGQGTLVTVSSEPKSCDKTHTCPPCPAPELLGGPSVFLFPPKPKDTLMISRTPEVTCVVVDVSHEDPEVKFNWYVDGVEVHNAKTKPREEQYNSTYRVVSVLTVLHQDWLNGKEYKCKVSNKALPAPIEKTISKAKGQPREPQVYTLPPSRDELTKNQVSLTCLVKGFYPSDIAVEWESNGQPENNYKTTPPVLDSDGSFFLYSKLTVDKSRWQQGNVFSCSVMHEALHNHYTQKSLSLSPG

SEQ ID NO: 104 - protein, 350 aa, Artificial Sequence
  Amino acid sequence of Anti-C18.2-32-Fc
QVQLVESGGGLVQPGGSLRLSCAASGEISSDAMAWYRQAPGKQRELVAGMTRGGSTNYADSVKGRFTISRDFAKNTVDLQMNSLKPEDTAVYYCNAEIYTGTFYPRSYWGQGTLVTVSSEPKSCDKTHTCPPCPAPELLGGPSVFLFPPKPKDTLMISRTPEVTCVVVDVSHEDPEVKFNWYVDGVEVHNAKTKPREEQYNSTYRVVSVLTVLHQDWLNGKEYKCKVSNKALPAPIEKTISKAKGQPREPQVYTLPPSRDELTKNQVSLTCLVKGFYPSDIAVEWESNGQPENNYKTTPPVLDSDGSFFLYSKLTVDKSRWQQGNVFSCSVMHEALHNHYTQKSLSLSPG

SEQ ID NO: 105 - protein, 352 aa, Artificial Sequence
  Amino acid sequence of Anti-C18.2-69-Fc
QVQLVESGGGLVQPGGSLRLSCAASGSIFSIPVMTWYRQALGKEREFVAGISKGGTSNYADSVKGRFTVSRDNAKNTVYLQMNSLKSEDTAVYYCNAQASSFGWMPLSDYWGQGTLVTVSSEPKSCDKTHTCPPCPAPELLGGPSVFLFPPKPKDTLMISRTPEVTCVVVDVSHEDPEVKFNWYVDGVEVHNAKTKPREEQYNSTYRVVSVLTVLHQDWLNGKEYKCKVSNKALPAPIEKTISKAKGQPREPQVYTLPPSRDELTKNQVSLTCLVKGFYPSDIAVEWESNGQPENNYKTTPPVLDSDGSFFLYSKLTVDKSRWQQGNVFSCSVMHEALHNHYTQKSLSLSPG

SEQ ID NO: 106 - protein, 352 aa, Artificial Sequence
  Amino acid sequence of Anti-C18.2-hu6V2-Fc
QVQLVESGGGLVQPGGSLRLSCAASGGIFSIGVMGWVRQAPGKGLEWVATITSRGSTNYADSVKGRFTISRDNSKNTLYLQMNSLRAEDTAVYYCYADLIRPGDFYGMDYWGQGTLVTVSSEPKSCDKTHTCPPCPAPELLGGPSVFLFPPKPKDTLMISRTPEVTCVVVDVSHEDPEVKFNWYVDGVEVHNAKTKPREEQYNSTYRVVSVLTVLHQDWLNGKEYKCKVSNKALPAPIEKTISKAKGQPREPQVYTLPPSRDELTKNQVSLTCLVKGFYPSDIAVEWESNGQPENNYKTTPPVLDSDGSFFLYSKLTVDKSRWQQGNVFSCSVMHEALHNHYTQKSLSLSPG

SEQ ID NO: 107 - protein, 352 aa, Artificial Sequence
  Amino acid sequence of Anti-C18.2-hu6V3-Fc
QVQLVESGGGLVQPGGSLRLSCAASGGIFSIGVMGWYRQAPGKGLELVATITSRGSTNYADSVKGRFTISRDNSKNTLYLQMNSLRAEDTAVYYCYADLIRPGDFYGMDYWGQGTLVTVSSEPKSCDKTHTCPPCPAPELLGGPSVFLFPPKPKDTLMISRTPEVTCVVVDVSHEDPEVKFNWYVDGVEVHNAKTKPREEQYNSTYRVVSVLTVLHQDWLNGKEYKCKVSNKALPAPIEKTISKAKGQPREPQVYTLPPSRDELTKNQVSLTCLVKGFYPSDIAVEWESNGQPENNYKTTPPVLDSDGSFFLYSKLTVDKSRWQQGNVFSCSVMHEALHNHYTQKSLSLSPG

SEQ ID NO: 108 - protein, 351 aa, Artificial Sequence
  Amino acid sequence of Anti-C18.2-hu19V1-Fc
QVQLVESGGGLVQPGGSLRLSCAASGVDISSDVMAWYRQAPGKQREFVSGLTRGGSINYADSVKGRFTISRDNSKNTLYLQMNSLRAEDTAVYYCNAEIYTGTFYPRSYWGQGTLVTVSSEPKSCDKTHTCPPCPAPELLGGPSVFLFPPKPKDTLMISRTPEVTCVVVDVSHEDPEVKFNWYVDGVEVHNAKTKPREEQYNSTYRVVSVLTVLHQDWLNGKEYKCKVSNKALPAPIEKTISKAKGQPREPQVYTLPPSRDELTKNQVSLTCLVKGFYPSDIAVEWESNGQPENNYKTTPPVLDSDGSFFLYSKLTVDKSRWQQGNVFSCSVMHEALHNHYTQKSLSLSPG

SEQ ID NO: 109 - protein, 351 aa, Artificial Sequence
  Amino acid sequence of Anti-C18.2-hu19V3-Fc
QVQLVESGGGLVQPGGSLRLSCAASGVDISSDVMAWYRQAPGKGLEFVSGLTRGGSINYADSVKGRFTISRDNSKNTLYLQMNSLRAEDTAVYYCNAEIYTGTFYPRSYWGQGTLVTVSSEPKSCDKTHTCPPCPAPELLGGPSVFLFPPKPKDTLMISRTPEVTCVVVDVSHEDPEVKFNWYVDGVEVHNAKTKPREEQYNSTYRVVSVLTVLHQDWLNGKEYKCKVSNKALPAPIEKTISKAKGQPREPQVYTLPPSRDELTKNQVSLTCLVKGFYPSDIAVEWESNGQPENNYKTTPPVLDSDGSFFLYSKLTVDKSRWQQGNVFSCSVMHEALHNHYTQKSLSLSPG

SEQ ID NO: 110 - DNA, 18 bp, Artificial Sequence
  Upstream primer of the first round of PCR
cttggtggtcctggctgc

SEQ ID NO: 111 - DNA, 23 bp, Artificial Sequence
  Downstream primer of the first round of PCR
ggtacgtgctgttgaactgttcc

SEQ ID NO: 112 - DNA, 47 bp, Artificial Sequence
  Upstream primer of the second round of PCR
catgccatgactgtggcccaggcggcccagktgcagctcgtggagtc

SEQ ID NO: 113 - DNA, 51 bp, Artificial Sequence
  Downstream primer of the second round of PCR
catgccatgactcgcggccggcctggccatgggggtcttcgctgtggtgcg

SEQ ID NO: 114 - DNA, 52 bp, Artificial Sequence
  Downstream primer of the second round of PCR
catgccatgactcgcggccggcctggccgtcttgtggttttggtgtcttggg

SEQ ID NO: 115 - DNA, 51 bp, Artificial Sequence
  Upstream primer
gtttaactttaagaaggagatatacatatgcaggtgcagctcgtggagtct

SEQ ID NO: 116 - DNA, 58 bp, Artificial Sequence
  Downstream primer
ggccgcaagcttgtcgacggagctcgaattcttactaatggtgatggtgatggtgctg

SEQ ID NO: 117 - DNA, 53 bp, Artificial Sequence
  Upstream primer
gtgctgctgctgtgggtgccaggatccaccgggcaggtgcagctcgtggagtc

SEQ ID NO: 118 - DNA, 45 bp, Artificial Sequence
  Downstream primer
gcaggacttgggctcagaagacacggtgaccagggtcccctggcc

SEQ ID NO: 119 - DNA, 1056 bp, Artificial Sequence
  Nucleic acid sequence of the isolated polynucleotide
caggtgcagctcgtggagtctgggggaggcttggtgcagcctggggggtctctgagactctcctgtgcagcctctgggggcatcttcagtatcggtgtcatgggctggtaccgccaggctccagggaagcagcgcgaattggtcgcgactattactagtcgtggtagcacaaactatgcagactccgtgaagggccgattcaccatctccggagacaacgccaagaacacggtgtatctacaaatgaacaacctgaaacctgaggacacggccgtctattactgttatgcagatctcataagacccggtgatttctacggcatggactactggggccaggggaccctggtcaccgtgtcttctgagcccaagtcctgcgacaaaactcacacatgcccaccgtgcccagcacctgaactcctgggtggaccgtcagtcttcctcttccccccaaaacccaaggacaccctcatgatctcccggacccctgaggtcacatgcgtggtggtggacgtgagccacgaagaccctgaggtcaagttcaactggtacgtggacggcgtggaggtgcataatgccaagacaaagccgcgggaggagcagtacaatagcacgtaccgtgtggtcagcgtcctcaccgtcctgcaccaggactggctgaatggcaaggagtacaagtgcaaggtctccaacaaagccctcccagcccccatcgagaaaaccatctccaaagccaaagggcagccccgagaaccacaggtgtacaccctgcccccatcccgggatgagctgaccaagaaccaggtcagcctgacctgcctggtcaaaggcttctatcccagcgacatcgccgtggagtgggagagcaatgggcagccggagaacaactacaagaccacgcctcccgtgctggactccgacggctccttcttcctctatagcaagctcaccgtggacaagagcaggtggcagcaggggaacgtcttctcatgctccgtgatgcatgaggctctgcacaaccactacacgcagaagagcctctccctgtctccgggt

SEQ ID NO: 120 - DNA, 1059 bp, Artificial Sequence
  Nucleic acid sequence of the isolated polynucleotide
caggtgcagctcgtggagtctgggggaggcttggtgcagcctggggggtctctgagactctcctgtgcagcctctggaagcatcttccttatcaatgccatgggctggtaccgccaggctccagggaagcagcgcgagttggtcgcagttattactagaggtggtagcgcaaactatacagactccgtgaagggccgattcaccatctccagagacaacgccaagaatacggtgtatctgcaaatgaacagcctgaaacctgaggacacggccgtctattactgtaatgcagatttgaacttaaggagcgacccctttaaatggtatacgttttggggccaggggaccctggtcaccgtgtcttctgagcccaagtcctgcgacaaaactcacacatgcccaccgtgcccagcacctgaactcctgggtggaccgtcagtcttcctcttccccccaaaacccaaggacaccctcatgatctcccggacccctgaggtcacatgcgtggtggtggacgtgagccacgaagaccctgaggtcaagttcaactggtacgtggacggcgtggaggtgcataatgccaagacaaagccgcgggaggagcagtacaatagcacgtaccgtgtggtcagcgtcctcaccgtcctgcaccaggactggctgaatggcaaggagtacaagtgcaaggtctccaacaaagccctcccagcccccatcgagaaaaccatctccaaagccaaagggcagccccgagaaccacaggtgtacaccctgcccccatcccgggatgagctgaccaagaaccaggtcagcctgacctgcctggtcaaaggcttctatcccagcgacatcgccgtggagtgggagagcaatgggcagccggagaacaactacaagaccacgcctcccgtgctggactccgacggctccttcttcctctatagcaagctcaccgtggacaagagcaggtggcagcaggggaacgtcttctcatgctccgtgatgcatgaggctctgcacaaccactacacgcagaagagcctctccctgtctccgggt

SEQ ID NO: 121 - DNA, 1056 bp, Artificial Sequence
  Nucleic acid sequence of the isolated polynucleotide
caggtgcagctcgtggagtctgggggaggcttggtgcagcctggggggtctctaagactctcctgtacagcctctggaagcatcttcaggatcgatggcatgcattggtaccgccaggctccagggaagcagcgcgagttggtcgcaagtattactcctagtggtatcacccactatgcagactccgtgaagggccgattcaccatctccagagacatcgccaagaaaatgcagtatctgcaaatgaacagcctgaaacctgaggacacggccgtctattactgtaatgcacacctcgtcaaagttggcggagtttggagtgatgagtactggggccaggggaccctggtcaccgtgtcttctgagcccaagtcctgcgacaaaactcacacatgcccaccgtgcccagcacctgaactcctgggtggaccgtcagtcttcctcttccccccaaaacccaaggacaccctcatgatctcccggacccctgaggtcacatgcgtggtggtggacgtgagccacgaagaccctgaggtcaagttcaactggtacgtggacggcgtggaggtgcataatgccaagacaaagccgcgggaggagcagtacaatagcacgtaccgtgtggtcagcgtcctcaccgtcctgcaccaggactggctgaatggcaaggagtacaagtgcaaggtctccaacaaagccctcccagcccccatcgagaaaaccatctccaaagccaaagggcagccccgagaaccacaggtgtacaccctgcccccatcccgggatgagctgaccaagaaccaggtcagcctgacctgcctggtcaaaggcttctatcccagcgacatcgccgtggagtgggagagcaatgggcagccggagaacaactacaagaccacgcctcccgtgctggactccgacggctccttcttcctctatagcaagctcaccgtggacaagagcaggtggcagcaggggaacgtcttctcatgctccgtgatgcatgaggctctgcacaaccactacacgcagaagagcctctccctgtctccgggt

SEQ ID NO: 122 - DNA, 1053 bp, Artificial Sequence
  Nucleic acid sequence of the isolated polynucleotide
caggtgcagctcgtggagtctgggggaggcttggtgcagcctggggggtctctgagactctcctgtgcagcctctggagtcgacatcagtagcgatgtcatggcctggtaccgccaggctccagggaagcagcgcgagtttgtctcaggccttactagaggtggtagcataaactatgcagactccgtgaagggccgattcaccatctccagagacttcgccaagaacacggtagatctgcaaatgaacagcctgaaacctgaggacacggccgtctattactgtaatgcagaaatctatactggtactttctacccgaggtcctactggggccaggggaccctggtcaccgtgtcttctgagcccaagtcctgcgacaaaactcacacatgcccaccgtgcccagcacctgaactcctgggtggaccgtcagtcttcctcttccccccaaaacccaaggacaccctcatgatctcccggacccctgaggtcacatgcgtggtggtggacgtgagccacgaagaccctgaggtcaagttcaactggtacgtggacggcgtggaggtgcataatgccaagacaaagccgcgggaggagcagtacaatagcacgtaccgtgtggtcagcgtcctcaccgtcctgcaccaggactggctgaatggcaaggagtacaagtgcaaggtctccaacaaagccctcccagcccccatcgagaaaaccatctccaaagccaaagggcagccccgagaaccacaggtgtacaccctgcccccatcccgggatgagctgaccaagaaccaggtcagcctgacctgcctggtcaaaggcttctatcccagcgacatcgccgtggagtgggagagcaatgggcagccggagaacaactacaagaccacgcctcccgtgctggactccgacggctccttcttcctctatagcaagctcaccgtggacaagagcaggtggcagcaggggaacgtcttctcatgctccgtgatgcatgaggctctgcacaaccactacacgcagaagagcctctccctgtctccgggt

SEQ ID NO: 123 - DNA, 1059 bp, Artificial Sequence
  Nucleic acid sequence of the isolated polynucleotide
caggtgcagctcgtggagtctgggggaggattggtgcagcctggggggtctctgagactctcctgtgcagcctctggaagcatcttcagtatcaatgccatgggctggtaccgccaggctccagggaagcagcgcgagttggtcgcagcaattacttttggtggtggtagcacaaactatgcagactccgtgaagggccgattcaccatctccagagacaacgccaagaacacggtgtatctgcaaatgaacagcctgaaacctgaggacacggccgtctattactgtaatgcagatctcctggtaggtggatttccgaggcggaatgtctactggggccaggggaccctggtcaccgtgtcttctgagcccaagtcctgcgacaaaactcacacatgcccaccgtgcccagcacctgaactcctgggtggaccgtcagtcttcctcttccccccaaaacccaaggacaccctcatgatctcccggacccctgaggtcacatgcgtggtggtggacgtgagccacgaagaccctgaggtcaagttcaactggtacgtggacggcgtggaggtgcataatgccaagacaaagccgcgggaggagcagtacaatagcacgtaccgtgtggtcagcgtcctcaccgtcctgcaccaggactggctgaatggcaaggagtacaagtgcaaggtctccaacaaagccctcccagcccccatcgagaaaaccatctccaaagccaaagggcagccccgagaaccacaggtgtacaccctgcccccatcccgggatgagctgaccaagaaccaggtcagcctgacctgcctggtcaaaggcttctatcccagcgacatcgccgtggagtgggagagcaatgggcagccggagaacaactacaagaccacgcctcccgtgctggactccgacggctccttcttcctctatagcaagctcaccgtggacaagagcaggtggcagcaggggaacgtcttctcatgctccgtgatgcatgaggctctgcacaaccactacacgcagaagagcctctccctgtctccgggt

SEQ ID NO: 124 - DNA, 1059 bp, Artificial Sequence
  Nucleic acid sequence of the isolated polynucleotide
caggtgcagctcgtggagtctgggggaggtttggtgcagcctggggggtctctgagactctcctgtgcagcctctggaagcatcttcatgatcaatgtcatgggctggtaccgccaggctccagggaagcagcgcgagttggtcgcagttattactagaggtgctagcacaaactatgcagactccgtgaagggccgattcaccatctccagagacaacgccaagaatacggtctatctgcaaatgaacagcctgaaacctgaggacacggccgtctattactgtaatgcagatttgaacttagcgagcgacccctttaaatggtatacgtattggggccaggggaccctggtcaccgtgtcttctgagcccaagtcctgcgacaaaactcacacatgcccaccgtgcccagcacctgaactcctgggtggaccgtcagtcttcctcttccccccaaaacccaaggacaccctcatgatctcccggacccctgaggtcacatgcgtggtggtggacgtgagccacgaagaccctgaggtcaagttcaactggtacgtggacggcgtggaggtgcataatgccaagacaaagccgcgggaggagcagtacaatagcacgtaccgtgtggtcagcgtcctcaccgtcctgcaccaggactggctgaatggcaaggagtacaagtgcaaggtctccaacaaagccctcccagcccccatcgagaaaaccatctccaaagccaaagggcagccccgagaaccacaggtgtacaccctgcccccatcccgggatgagctgaccaagaaccaggtcagcctgacctgcctggtcaaaggcttctatcccagcgacatcgccgtggagtgggagagcaatgggcagccggagaacaactacaagaccacgcctcccgtgctggactccgacggctccttcttcctctatagcaagctcaccgtggacaagagcaggtggcagcaggggaacgtcttctcatgctccgtgatgcatgaggctctgcacaaccactacacgcagaagagcctctccctgtctccgggt

SEQ ID NO: 125 - DNA, 1050 bp, Artificial Sequence
  Nucleic acid sequence of the isolated polynucleotide
caggtgcagctcgtggagtctgggggaggcttggtgcagcctggggggtctctgagactctcctgtgcagcctctggagaaatcagtagcgatgccatggcctggtaccgccaggctccagggaaacagcgcgagttggtcgcaggtatgactagaggtggtagcacaaactatgcagactccgtgaagggccgattcaccatctccagagacttcgccaagaacacggtagatctgcaaatgaacagcctgaaacctgaggacacggccgtctattactgtaatgcagaaatctatactggtactttctacccgaggtcctactggggccaggggaccctggtcaccgtgtcttctgagcccaagtcctgcgacaaaactcacacatgcccaccgtgcccagcacctgaactcctgggtggaccgtcagtcttcctcttccccccaaaacccaaggacaccctcatgatctcccggacccctgaggtcacatgcgtggtggtggacgtgagccacgaagaccctgaggtcaagttcaactggtacgtggacggcgtggaggtgcataatgccaagacaaagccgcgggaggagcagtacaatagcacgtaccgtgtggtcagcgtcctcaccgtcctgcaccaggactggctgaatggcaaggagtacaagtgcaaggtctccaacaaagccctcccagcccccatcgagaaaaccatctccaaagccaaagggcagccccgagaaccacaggtgtacaccctgcccccatcccgggatgagctgaccaagaaccaggtcagcctgacctgcctggtcaaaggcttctatcccagcgacatcgccgtggagtgggagagcaatgggcagccggagaacaactacaagaccacgcctcccgtgctggactccgacggctccttcttcctctatagcaagctcaccgtggacaagagcaggtggcagcaggggaacgtcttctcatgctccgtgatgcatgaggctctgcacaaccactacacgcagaagagcctctccctgtctccgggt

SEQ ID NO: 126 - DNA, 1056 bp, Artificial Sequence
  Nucleic acid sequence of the isolated polynucleotide
caggtgcagctcgtggagtccgggggaggcttggtgcagcctggggggtctctgagactctcctgtgcagcctctggaagcatcttcagtatccctgtcatgacctggtaccgccaggctctagggaaagagcgcgagttcgtcgcaggtattagtaagggtggtacctcgaactatgcagactccgtgaagggccgattcaccgtctccagagacaacgccaagaacacggtgtatctgcaaatgaacagcctgaaatcagaggacacggccgtctattactgcaatgcacaagcttcttcgttcggttggatgcccctctctgactactggggccaggggaccctggtcaccgtgtcttctgagcccaagtcctgcgacaaaactcacacatgcccaccgtgcccagcacctgaactcctgggtggaccgtcagtcttcctcttccccccaaaacccaaggacaccctcatgatctcccggacccctgaggtcacatgcgtggtggtggacgtgagccacgaagaccctgaggtcaagttcaactggtacgtggacggcgtggaggtgcataatgccaagacaaagccgcgggaggagcagtacaatagcacgtaccgtgtggtcagcgtcctcaccgtcctgcaccaggactggctgaatggcaaggagtacaagtgcaaggtctccaacaaagccctcccagcccccatcgagaaaaccatctccaaagccaaagggcagccccgagaaccacaggtgtacaccctgcccccatcccgggatgagctgaccaagaaccaggtcagcctgacctgcctggtcaaaggcttctatcccagcgacatcgccgtggagtgggagagcaatgggcagccggagaacaactacaagaccacgcctcccgtgctggactccgacggctccttcttcctctatagcaagctcaccgtggacaagagcaggtggcagcaggggaacgtcttctcatgctccgtgatgcatgaggctctgcacaaccactacacgcagaagagcctctccctgtctccgggt

SEQ ID NO: 127 - DNA, 1056 bp, Artificial Sequence
  Nucleic acid sequence of the isolated polynucleotide
caggtgcagctcgtggagtctgggggaggcttggtgcagcctggggggtctctgagactctcctgtgcagcctctgggggcatcttcagtatcggtgtcatgggctgggtgcgccaggctccagggaagggcctggagtgggtcgcgactattactagtcgtggtagcacaaactatgcagactccgtgaagggccgattcaccatctccagagacaacagcaagaacacgctgtatctacaaatgaacagcctgcgggccgaggacacggccgtctattactgttatgcagatctcataagacccggtgatttctacggcatggactactggggccaggggaccctggtcaccgtgtcttctgagcccaagtcctgcgacaaaactcacacatgcccaccgtgcccagcacctgaactcctgggtggaccgtcagtcttcctcttccccccaaaacccaaggacaccctcatgatctcccggacccctgaggtcacatgcgtggtggtggacgtgagccacgaagaccctgaggtcaagttcaactggtacgtggacggcgtggaggtgcataatgccaagacaaagccgcgggaggagcagtacaatagcacgtaccgtgtggtcagcgtcctcaccgtcctgcaccaggactggctgaatggcaaggagtacaagtgcaaggtctccaacaaagccctcccagcccccatcgagaaaaccatctccaaagccaaagggcagccccgagaaccacaggtgtacaccctgcccccatcccgggatgagctgaccaagaaccaggtcagcctgacctgcctggtcaaaggcttctatcccagcgacatcgccgtggagtgggagagcaatgggcagccggagaacaactacaagaccacgcctcccgtgctggactccgacggctccttcttcctctatagcaagctcaccgtggacaagagcaggtggcagcaggggaacgtcttctcatgctccgtgatgcatgaggctctgcacaaccactacacgcagaagagcctctccctgtctccgggt

SEQ ID NO: 128 - DNA, 1056 bp, Artificial Sequence
  Nucleic acid sequence of the isolated polynucleotide
caggtgcagctcgtggagtctgggggaggcttggtgcagcctggggggtctctgagactctcctgtgcagcctctgggggcatcttcagtatcggtgtcatgggctggtaccgccaggctccagggaagggcctggagctggtcgcgactattactagtcgtggtagcacaaactatgcagactccgtgaagggccgattcaccatctccagagacaacagcaagaacacgctgtatctacaaatgaacagcctgcgggccgaggacacggccgtctattactgttatgcagatctcataagacccggtgatttctacggcatggactactggggccaggggaccctggtcaccgtgtcttctgagcccaagtcctgcgacaaaactcacacatgcccaccgtgcccagcacctgaactcctgggtggaccgtcagtcttcctcttccccccaaaacccaaggacaccctcatgatctcccggacccctgaggtcacatgcgtggtggtggacgtgagccacgaagaccctgaggtcaagttcaactggtacgtggacggcgtggaggtgcataatgccaagacaaagccgcgggaggagcagtacaatagcacgtaccgtgtggtcagcgtcctcaccgtcctgcaccaggactggctgaatggcaaggagtacaagtgcaaggtctccaacaaagccctcccagcccccatcgagaaaaccatctccaaagccaaagggcagccccgagaaccacaggtgtacaccctgcccccatcccgggatgagctgaccaagaaccaggtcagcctgacctgcctggtcaaaggcttctatcccagcgacatcgccgtggagtgggagagcaatgggcagccggagaacaactacaagaccacgcctcccgtgctggactccgacggctccttcttcctctatagcaagctcaccgtggacaagagcaggtggcagcaggggaacgtcttctcatgctccgtgatgcatgaggctctgcacaaccactacacgcagaagagcctctccctgtctccgggt

SEQ ID NO: 129 - DNA, 1053 bp, Artificial Sequence
  Nucleic acid sequence of the isolated polynucleotide
caggtgcagctcgtggagtctgggggaggcttggtgcagcctggggggtctctgagactctcctgtgcagcctctggagtcgacatcagtagcgatgtcatggcctggtaccgccaggctccagggaagcagcgggagttcgtctcaggccttactagaggtggtagcataaactatgcagactccgtgaagggccgattcaccatctccagagacaacagcaagaacacgctgtacctgcaaatgaacagcctgagagccgaggacacggccgtctattactgtaatgcagaaatctatactggtactttctacccgaggtcctactggggccaggggaccctggtcaccgtgtcttctgagcccaagtcctgcgacaaaactcacacatgcccaccgtgcccagcacctgaactcctgggtggaccgtcagtcttcctcttccccccaaaacccaaggacaccctcatgatctcccggacccctgaggtcacatgcgtggtggtggacgtgagccacgaagaccctgaggtcaagttcaactggtacgtggacggcgtggaggtgcataatgccaagacaaagccgcgggaggagcagtacaatagcacgtaccgtgtggtcagcgtcctcaccgtcctgcaccaggactggctgaatggcaaggagtacaagtgcaaggtctccaacaaagccctcccagcccccatcgagaaaaccatctccaaagccaaagggcagccccgagaaccacaggtgtacaccctgcccccatcccgggatgagctgaccaagaaccaggtcagcctgacctgcctggtcaaaggcttctatcccagcgacatcgccgtggagtgggagagcaatgggcagccggagaacaactacaagaccacgcctcccgtgctggactccgacggctccttcttcctctatagcaagctcaccgtggacaagagcaggtggcagcaggggaacgtcttctcatgctccgtgatgcatgaggctctgcacaaccactacacgcagaagagcctctccctgtctccgggt

SEQ ID NO: 130 - DNA, 1053 bp, Artificial Sequence
  Nucleic acid sequence of the isolated polynucleotide
caggtgcagctcgtggagtctgggggaggcttggtgcagcctggggggtctctgagactctcctgtgcagcctctggagtcgacatcagtagcgatgtcatggcctggtaccgccaggctccagggaagggcctggagttcgtctcaggccttactagaggtggtagcataaactatgcagactccgtgaagggccgattcaccatctccagagacaacagcaagaacacgctgtacctgcaaatgaacagcctgagagccgaggacacggccgtctattactgtaatgcagaaatctatactggtactttctacccgaggtcctactggggccaggggaccctggtcaccgtgtcttctgagcccaagtcctgcgacaaaactcacacatgcccaccgtgcccagcacctgaactcctgggtggaccgtcagtcttcctcttccccccaaaacccaaggacaccctcatgatctcccggacccctgaggtcacatgcgtggtggtggacgtgagccacgaagaccctgaggtcaagttcaactggtacgtggacggcgtggaggtgcataatgccaagacaaagccgcgggaggagcagtacaatagcacgtaccgtgtggtcagcgtcctcaccgtcctgcaccaggactggctgaatggcaaggagtacaagtgcaaggtctccaacaaagccctcccagcccccatcgagaaaaccatctccaaagccaaagggcagccccgagaaccacaggtgtacaccctgcccccatcccgggatgagctgaccaagaaccaggtcagcctgacctgcctggtcaaaggcttctatcccagcgacatcgccgtggagtgggagagcaatgggcagccggagaacaactacaagaccacgcctcccgtgctggactccgacggctccttcttcctctatagcaagctcaccgtggacaagagcaggtggcagcaggggaacgtcttctcatgctccgtgatgcatgaggctctgcacaaccactacacgcagaagagcctctccctgtctccgggt

SEQ ID NO: 131 - protein, 124 aa, Artificial Sequence
  Amino acid sequence of anti-CD3 nanobody
EVQLVESGGGPVQAGGSLRLSCAASGRTYRGYSMGWFRQAPGKEREFVAAIVWSGGNTYYEDSVKGRFTISRDNAKNTMYLQMTSLKPEDSATYYCAAKIRPYIFKIAGQYDYWGQGTQVTVSS

SEQ ID NO: 132 - protein, 35 aa, Artificial Sequence
  GS sequence
GGGGSGGGGSGGGGSGGGGSGGGGSGGGGSGGGGS

SEQ ID NO: 133 - protein, 280 aa, Artificial Sequence
  Amino acid sequence of Anti-CLDN18×CD3-hu6V3
QVQLVESGGGLVQPGGSLRLSCAASGGIFSIGVMGWYRQAPGKGLELVATITSRGSTNYADSVKGRFTISRDNSKNTLYLQMNSLRAEDTAVYYCYADLIRPGDFYGMDYWGQGTLVTVSSGGGGSGGGGSGGGGSGGGGSGGGGSGGGGSGGGGSEVQLVESGGGPVQAGGSLRLSCAASGRTYRGYSMGWFRQAPGKEREFVAAIVWSGGNTYYEDSVKGRFTISRDNAKNTMYLQMTSLKPEDSATYYCAAKIRPYIFKIAGQYDYWGQGTQVTVSS

SEQ ID NO: 134 - protein, 279 aa, Artificial Sequence
  Amino acid sequence of Anti-CLDN18×CD3-hu19V3
QVQLVESGGGLVQPGGSLRLSCAASGVDISSDVMAWYRQAPGKGLEFVSGLTRGGSINYADSVKGRFTISRDNSKNTLYLQMNSLRAEDTAVYYCNAEIYTGTFYPRSYWGQGTLVTVSSGGGGSGGGGSGGGGSGGGGSGGGGSGGGGSGGGGSEVQLVESGGGPVQAGGSLRLSCAASGRTYRGYSMGWFRQAPGKEREFVAAIVWSGGNTYYEDSVKGRFTISRDNAKNTMYLQMTSLKPEDSATYYCAAKIRPYIFKIAGQYDYWGQGTQVTVSS

SEQ ID NO: 135 - protein, 226 aa, Artificial Sequence
  Amino acid sequence of CD8 hinge-CD28a-CD28b- CD3ζ
TTTPAPRPPTPAPTIASQPLSLRPEACRPAAGGAVHTRGLDFACDFWVLVVVGGVLACYSLLVTVAFIIFWVRSKRSRLLHSDYMNMTPRRPGPTRKHYQPYAPPRDFAAYRSRVKFSRSADAPAYQQGQNQLYNELNLGRREEYDVLDKRRGRDPEMGGKPQRRKNPQEGLYNELQKDKMAEAYSEIGMKGERRRGKGHDGLYQGLSTATKDTYDALHMQALPPR

SEQ ID NO: 136 - protein, 268 aa, Artificial Sequence
  Amino acid sequence of CD8 hinge-CD28a-CD28b-CD137- CD3ζ
TTTPAPRPPTPAPTIASQPLSLRPEACRPAAGGAVHTRGLDFACDFWVLVVVGGVLACYSLLVTVAFIIFWVRSKRSRLLHSDYMNMTPRRPGPTRKHYQPYAPPRDFAAYRSKRGRKKLLYIFKQPFMRPVQTTQEEDGCSCRFPEEEEGGCELRVKFSRSADAPAYQQGQNQLYNELNLGRREEYDVLDKRRGRDPEMGGKPQRRKNPQEGLYNELQKDKMAEAYSEIGMKGERRRGKGHDGLYQGLSTATKDTYDALHMQALPPR

SEQ ID NO: 137 - protein, 347 aa, Artificial Sequence
  Amino acid sequence of VHH(Anti-CLD18A2-hu6V3)-CD8 hinge-CD28a-CD28b- CD3ζ
QVQLVESGGGLVQPGGSLRLSCAASGGIFSIGVMGWYRQAPGKGLELVATITSRGSTNYADSVKGRFTISRDNSKNTLYLQMNSLRAEDTAVYYCYADLIRPGDFYGMDYWGQGTLVTVSSTTTPAPRPPTPAPTIASQPLSLRPEACRPAAGGAVHTRGLDFACDFWVLVVVGGVLACYSLLVTVAFIIFWVRSKRSRLLHSDYMNMTPRRPGPTRKHYQPYAPPRDFAAYRSRVKFSRSADAPAYQQGQNQLYNELNLGRREEYDVLDKRRGRDPEMGGKPQRRKNPQEGLYNELQKDKMAEAYSEIGMKGERRRGKGHDGLYQGLSTATKDTYDALHMQALPPR

SEQ ID NO: 138 - protein, 389 aa, Artificial Sequence
  Amino acid sequence of VHH(Anti-CLD18A2-hu6V3)-CD8 hinge-CD28a-CD28b-CD137-CD3ζ
QVQLVESGGGLVQPGGSLRLSCAASGGIFSIGVMGWYRQAPGKGLELVATITSRGSTNYADSVKGRFTISRDNSKNTLYLQMNSLRAEDTAVYYCYADLIRPGDFYGMDYWGQGTLVTVSSTTTPAPRPPTPAPTIASQPLSLRPEACRPAAGGAVHTRGLDFACDFWVLVVVGGVLACYSLLVTVAFIIFWVRSKRSRLLHSDYMNMTPRRPGPTRKHYQPYAPPRDFAAYRSKRGRKKLLYIFKQPFMRPVQTTQEEDGCSCRFPEEEEGGCELRVKFSRSADAPAYQQGQNQLYNELNLGRREEYDVLDKRRGRDPEMGGKPQRRKNPQEGLYNELQKDKMAEAYSEIGMKGERRRGKGHDGLYQGLSTATKDTYDALHMQALPPR

SEQ ID NO: 139 - protein, 346 aa, Artificial Sequence
  Amino acid sequence of VHH(Anti-CLD18A2-hu19V3)-CD8 hinge-CD28a-CD28b- CD3ζ
QVQLVESGGGLVQPGGSLRLSCAASGVDISSDVMAWYRQAPGKGLEFVSGLTRGGSINYADSVKGRFTISRDNSKNTLYLQMNSLRAEDTAVYYCNAEIYTGTFYPRSYWGQGTLVTVSSTTTPAPRPPTPAPTIASQPLSLRPEACRPAAGGAVHTRGLDFACDFWVLVVVGGVLACYSLLVTVAFIIFWVRSKRSRLLHSDYMNMTPRRPGPTRKHYQPYAPPRDFAAYRSRVKFSRSADAPAYQQGQNQLYNELNLGRREEYDVLDKRRGRDPEMGGKPQRRKNPQEGLYNELQKDKMAEAYSEIGMKGERRRGKGHDGLYQGLSTATKDTYDALHMQALPPR

SEQ ID NO: 140 - protein, 388 aa, Artificial Sequence
  Amino acid sequence of VHH(Anti-CLD18A2-hu19V3)-CD8 hinge-CD28a-CD28b-CD137-CD3ζ
QVQLVESGGGLVQPGGSLRLSCAASGVDISSDVMAWYRQAPGKGLEFVSGLTRGGSINYADSVKGRFTISRDNSKNTLYLQMNSLRAEDTAVYYCNAEIYTGTFYPRSYWGQGTLVTVSSTTTPAPRPPTPAPTIASQPLSLRPEACRPAAGGAVHTRGLDFACDFWVLVVVGGVLACYSLLVTVAFIIFWVRSKRSRLLHSDYMNMTPRRPGPTRKHYQPYAPPRDFAAYRSKRGRKKLLYIFKQPFMRPVQTTQEEDGCSCRFPEEEEGGCELRVKFSRSADAPAYQQGQNQLYNELNLGRREEYDVLDKRRGRDPEMGGKPQRRKNPQEGLYNELQKDKMAEAYSEIGMKGERRRGKGHDGLYQGLSTATKDTYDALHMQALPPR

SEQ ID NO: 141 - DNA, 1617 bp, Artificial Sequence
  Sequence containing a CD8 signal peptide and a CD8 hinge-CD28a-CD28b-CD3-T2A-egfp structure
ggatccaggcctaagcttacgcgtgccaccatggccttaccagtgaccgccttgctcctgccgctggccttgctgctccacgccgccaggccgctgcagcatcatcatcatcatcatcatatgaccacgacgccagcgccgcgaccaccaacaccggcgcccaccatcgcgtcgcagcccctgtccctgcgcccagaggcgtgtcggccagcggcggggggcgcagtgcacacgagggggctggacttcgcctgtgatttttgggtgctggtggtggttggtggagtcctggcttgctatagcttgctagtaacagtggcctttattattttctgggtgaggagtaagaggagcaggctcctgcacagtgactacatgaacatgactccccgccgccccgggccaacccgcaagcattaccagccctatgccccaccacgcgacttcgcagcctatcgctccagagtgaagttcagcaggagcgcagacgcccccgcgtaccagcagggccagaaccagctctataacgaactcaatctaggacgaagagaggagtacgatgttttggacaagagacgtggccgggaccctgagatggggggaaagccgcagagaaggaagaaccctcaggaaggcctgtacaatgaactccagaaagataagatggcggaggcctacagtgagattgggatgaaaggcgagcgcagaaggggcaaggggcacgatggcctttaccagggtctcagtacagccaccaaggacacctacgacgcccttcacatgcaggccctgccccctcgcggaagcggagagggcagaggaagtctgctaacatgcggtgacgtcgaggagaatcctggacctatggtgagcaagggcgaggagctgttcaccggggtggtgcccatcctggtcgagctggacggcgacgtaaacggccacaagttcagcgtgtccggcgagggcgagggcgatgccacctacggcaagctgaccctgaagttcatctgcaccaccggcaagctgcccgtgccctggcccaccctcgtgaccaccctgacctacggcgtgcagtgcttcagccgctaccccgaccacatgaagcagcacgacttcttcaagtccgccatgcccgaaggctacgtccaggagcgcaccatcttcttcaaggacgacggcaactacaagacccgcgccgaggtgaagttcgagggcgacaccctggtgaaccgcatcgagctgaagggcatcgacttcaaggaggacggcaacatcctggggcacaagctggagtacaactacaacagccacaacgtctatatcatggccgacaagcagaagaacggcatcaaggtgaacttcaagatccgccacaacatcgaggacggcagcgtgcagctcgccgaccactaccagcagaacacccccatcggcgacggccccgtgctgctgcccgacaaccactacctgagcacccagtccgccctgagcaaagaccccaacgagaagcgcgatcacatggtcctgctggagttcgtgaccgccgccgggatcactctcggcatggacgagctgtacaagtgataagtcgacctcgagggaattccgataatcaac

SEQ ID NO: 142 - DNA, 1743 bp, Artificial Sequence
  Sequence containing a CD8 signal peptide and a CD8 hinge-CD28a-CD28b-CD137-CD3-T2A-egfp
ggatccaggcctaagcttacgcgtgccaccatggccttaccagtgaccgccttgctcctgccgctggccttgctgctccacgccgccaggccgctgcagcatcatcatcatcatcatcatatgaccacgacgccagcgccgcgaccaccaacaccggcgcccaccatcgcgtcgcagcccctgtccctgcgcccagaggcgtgtcggccagcggcggggggcgcagtgcacacgagggggctggacttcgcctgtgatttttgggtgctggtggtggttggtggagtcctggcttgctatagcttgctagtaacagtggcctttattattttctgggtgaggagtaagaggagcaggctcctgcacagtgactacatgaacatgactccccgccgccccgggccaacccgcaagcattaccagccctatgccccaccacgcgacttcgcagcctatcgctccaaacggggcagaaagaaactcctgtatatattcaaacaaccatttatgagaccagtacaaactactcaagaggaagatggctgtagctgccgatttccagaagaagaagaaggaggatgtgaactgagagtgaagttcagcaggagcgcagacgcccccgcgtaccagcagggccagaaccagctctataacgaactcaatctaggacgaagagaggagtacgatgttttggacaagagacgtggccgggaccctgagatggggggaaagccgcagagaaggaagaaccctcaggaaggcctgtacaatgaactccagaaagataagatggcggaggcctacagtgagattgggatgaaaggcgagcgcagaaggggcaaggggcacgatggcctttaccagggtctcagtacagccaccaaggacacctacgacgcccttcacatgcaggccctgccccctcgcggaagcggagagggcagaggaagtctgctaacatgcggtgacgtcgaggagaatcctggacctatggtgagcaagggcgaggagctgttcaccggggtggtgcccatcctggtcgagctggacggcgacgtaaacggccacaagttcagcgtgtccggcgagggcgagggcgatgccacctacggcaagctgaccctgaagttcatctgcaccaccggcaagctgcccgtgccctggcccaccctcgtgaccaccctgacctacggcgtgcagtgcttcagccgctaccccgaccacatgaagcagcacgacttcttcaagtccgccatgcccgaaggctacgtccaggagcgcaccatcttcttcaaggacgacggcaactacaagacccgcgccgaggtgaagttcgagggcgacaccctggtgaaccgcatcgagctgaagggcatcgacttcaaggaggacggcaacatcctggggcacaagctggagtacaactacaacagccacaacgtctatatcatggccgacaagcagaagaacggcatcaaggtgaacttcaagatccgccacaacatcgaggacggcagcgtgcagctcgccgaccactaccagcagaacacccccatcggcgacggccccgtgctgctgcccgacaaccactacctgagcacccagtccgccctgagcaaagaccccaacgagaagcgcgatcacatggtcctgctggagttcgtgaccgccgccgggatcactctcggcatggacgagctgtacaagtgataagtcgacctcgagggaattccgataatcaac

SEQ ID NO: 143 - DNA, 49 bp, Artificial Sequence
  Forward primer
cttgctgctccacgccgccaggccgcaggtgcagctcgtggagtctggg

SEQ ID NO: 144 - DNA, 50 bp, Artificial Sequence
  Reverse primer
ggtcgcggcgctggcgtcgtggtagaagacacggtgaccagggtcccctg